European Patent Specification EP 3 814 471 B1, published March 5, 2025. Title: Mittel enthaltend Polyesterase I. Applicant: Henkel AG & Co. KGaA. The sequence listing filed with the application follows.

SEQUENCE LISTING (2 sequences)

SEQ ID NO: 1 - protein, 262 aa, Thermomonospora curvata
AANPYQRGPNPTEASITAARGPFNTAEITVSRLSVSGFGGGKIYYPTTTSEGTFGAIAISPGFTAYWSSLEWLGHRLASQGFVVIGIETNTTLDQPDQRGQQLLAALDYLTQRSAVRDRVDASRLAVAGHSMGGGGSLEAAKARTSLKAAIPLAPWNLDKTWPEVRTPTLIIGGELDAVAPVATHSIPFYNSLSNAPEKAYLELDNASHFFPNITNTQMAKYMIAWMKRFIDDDTRYTQFLCPPPSTGLLSDFSDARFTCPM

SEQ ID NO: 2 - protein, 292 aa, Thermomonospora curvata
MKRTLKRALSLLPAAALAASALVAASPAQAAANPYQRGPNPTEASITAARGPFNTAEITVSRLSVSGFGGGKIYYPTTTSEGTFGAIAISPGFTAYWSSLEWLGHRLASQGFVVIGIETNTTLDQPDQRGQQLLAALDYLTQRSAVRDRVDASRLAVAGHSMGGGGSLEAAKARTSLKAAIPLAPWNLDKTWPEVRTPTLIIGGELDAVAPVATHSIPFYNSLSNAPEKAYLELDNASHFFPNITNTQMAKYMIAWMKRFIDDDTRYTQFLCPPPSTGLLSDFSDARFTCPM